European Patent Application EP 4 279 507 A1, published November 22, 2023. Title: CD73-BINDING PROTEIN AND USE THEREOF. Applicant: SHANGHAI HUAOTA BIOPHARMACEUTICAL CO., LTD.;HUABO BIOPHARM (SHANGHAI) CO., LTD. The sequence listing filed with the application follows.

SEQUENCE LISTING (55 sequences)

SEQ ID NO: 1 - protein, 14 aa, Artificial Sequence
  HCDR3
ARYYGSDYEWYFDV

SEQ ID NO: 2 - protein, 8 aa, Artificial Sequence
  HCDR2
IHPNSGST

SEQ ID NO: 3 - protein, 8 aa, Artificial Sequence
  HCDR1
GYTFTSYW

SEQ ID NO: 4 - protein, 9 aa, Artificial Sequence
  LCDR3
LQHWNYPYT

SEQ ID NO: 5 - protein, 3 aa, Artificial Sequence
  LCDR2
LAS

SEQ ID NO: 6 - protein, 6 aa, Artificial Sequence
  LCDR1
QNVRTA

SEQ ID NO: 7 - protein, 25 aa, Artificial Sequence
  900567(124A9) H-FR1
QVQLQQPGAELVKPGASVKLSCKAS

SEQ ID NO: 8 - protein, 17 aa, Artificial Sequence
  900567(124A9) H-FR2
IHWVKQRPGQGLDWIGM

SEQ ID NO: 9 - protein, 38 aa, Artificial Sequence
  900567(124A9) H-FR3
YYNEKFKSKATLTVDKSSSTAYMQLSSLTSEDSAVYYC

SEQ ID NO: 10 - protein, 11 aa, Artificial Sequence
  900567(124A9) H-FR4
WGTGTTVTVSS

SEQ ID NO: 11 - protein, 26 aa, Artificial Sequence
  900567(124A9) L-FR1
DIVMTQSQKFMSTSVGDRVSITCKAS

SEQ ID NO: 12 - protein, 17 aa, Artificial Sequence
  900567(124A9) L-FR2
VVWYQQNPGQSPKALIY

SEQ ID NO: 13 - protein, 36 aa, Artificial Sequence
  900567(124A9) L-FR3
NRHTGVPDRFTGSGSGTDFTLTISNVHSEDLADYFC

SEQ ID NO: 14 - protein, 10 aa, Artificial Sequence
  900567(124A9) L-FR4
FGGGTKLEIK

SEQ ID NO: 15 - protein, 25 aa, Artificial Sequence
  H-FR1 of 900725 900726
QVQLVQSGAEVKKPGASVKLSCKAS

SEQ ID NO: 16 - protein, 17 aa, Artificial Sequence
  H-FR2 of 900725 900726 900727 900728
IHWVRQAPGQGLEWIGM

SEQ ID NO: 17 - protein, 38 aa, Artificial Sequence
  H-FR3 900725 900726
YYNEKFKGRATLTVDKSTSTAYMELSSLRSEDTAVYYC

SEQ ID NO: 18 - protein, 11 aa, Artificial Sequence
  H-FR4 of 900725 900726 900727 900728
WGQGTTVTVSS

SEQ ID NO: 19 - protein, 26 aa, Artificial Sequence
  L-FR1 of 900725 900727
DIQMTQSPSSMSASVGDRVTITCKAS

SEQ ID NO: 20 - protein, 17 aa, Artificial Sequence
  L-FR2 of 900725 900726 900727 900728
VVWYQQKPGKAPKALIY

SEQ ID NO: 21 - protein, 36 aa, Artificial Sequence
  L-FR3 of 900725 900727
NRHTGVPDRFSGSGSGTDFTLTISSLQPEDFATYFC

SEQ ID NO: 22 - protein, 10 aa, Artificial Sequence
  L-FR4 of 900725 900726 900727 900728
FGQGTKLEIK

SEQ ID NO: 23 - protein, 25 aa, Artificial Sequence [sequence omitted]

SEQ ID NO: 24 - protein, 38 aa, Artificial Sequence
  900727 H-FR3
YYAQKFQGRVTITVDKSTSTAYMELSSLRSEDTAVYYC

SEQ ID NO: 25 - protein, 26 aa, Artificial Sequence [sequence omitted]

SEQ ID NO: 26 - protein, 36 aa, Artificial Sequence
  L-FR3 of 900726 900728
NRHTGVPDRFSGSGSGTDFTLTISSLQPEDFATYYC

SEQ ID NO: 27 - protein, 38 aa, Artificial Sequence
  900728 H-FR3
YYNEKFQGRVTMTVDKSTSTAYMELSSLRSEDTAVYYC

SEQ ID NO: 28 - protein, 121 aa, Artificial Sequence
  900567(124A9) VH
QVQLQQPGAELVKPGASVKLSCKASGYTFTSYWIHWVKQRPGQGLDWIGMIHPNSGSTYYNEKFKSKATLTVDKSSSTAYMQLSSLTSEDSAVYYCARYYGSDYEWYFDVWGTGTTVTVSS

SEQ ID NO: 29 - protein, 107 aa, Artificial Sequence
  900567(124A9) VL
DIVMTQSQKFMSTSVGDRVSITCKASQNVRTAVVWYQQNPGQSPKALIYLASNRHTGVPDRFTGSGSGTDFTLTISNVHSEDLADYFCLQHWNYPYTFGGGTKLEIK

SEQ ID NO: 30 - protein, 121 aa, Artificial Sequence
  VH of 900725 900726
QVQLVQSGAEVKKPGASVKLSCKASGYTFTSYWIHWVRQAPGQGLEWIGMIHPNSGSTYYNEKFKGRATLTVDKSTSTAYMELSSLRSEDTAVYYCARYYGSDYEWYFDVWGQGTTVTVSS

SEQ ID NO: 31 - protein, 107 aa, Artificial Sequence
  VL of 900725 900727
DIQMTQSPSSMSASVGDRVTITCKASQNVRTAVVWYQQKPGKAPKALIYLASNRHTGVPDRFSGSGSGTDFTLTISSLQPEDFATYFCLQHWNYPYTFGQGTKLEIK

SEQ ID NO: 32 - protein, 121 aa, Artificial Sequence
  900727 VH
QVQLVQSGAEVKKPGASVKVSCKASGYTFTSYWIHWVRQAPGQGLEWIGMIHPNSGSTYYAQKFQGRVTITVDKSTSTAYMELSSLRSEDTAVYYCARYYGSDYEWYFDVWGQGTTVTVSS

SEQ ID NO: 33 - protein, 107 aa, Artificial Sequence
  VL of 900726 900728
DIQMTQSPSSLSASVGDRVTITCKASQNVRTAVVWYQQKPGKAPKALIYLASNRHTGVPDRFSGSGSGTDFTLTISSLQPEDFATYYCLQHWNYPYTFGQGTKLEIK

SEQ ID NO: 34 - protein, 121 aa, Artificial Sequence
  900728 VH
QVQLVQSGAEVKKPGASVKVSCKASGYTFTSYWIHWVRQAPGQGLEWIGMIHPNSGSTYYNEKFQGRVTMTVDKSTSTAYMELSSLRSEDTAVYYCARYYGSDYEWYFDVWGQGTTVTVSS

SEQ ID NO: 35 - protein, 121 aa, Artificial Sequence
  900584 VH
QVQVQQPGTELVKPGASVKLSCKASGYTFTGYWMHWVKQRPGQGLEWIGMIHPNSGSTYYNEKFKSKATLTVDRSSSTAYMQLSSLSSEDSAVYYCARYYGTTYEWYFDVWGTGTTVTVSS

SEQ ID NO: 36 - protein, 107 aa, Artificial Sequence
  900584 VL
DIQMTQTTSSLSASLGDRVTISCRASQDISNYLNWYQQKPDGTVKPLIYYTSSLHSGVPSRFSGSGSGTDYSLTISDLEHEDIATYFCQQGYTLPFTFGGGTKLEIK

SEQ ID NO: 37 - protein, 329 aa, Artificial Sequence
  constant region of heavy chain
ASTKGPSVFPLAPSSKSTSGGTAALGCLVKDYFPEPVTVSWNSGALTSGVHTFPAVLQSSGLYSLSSVVTVPSSSLGTQTYICNVNHKPSNTKVDKRVEPKSCDKTHTCPPCPAPEAAGGPSVFLFPPKPKDTLMISRTPEVTCVVVDVSHEDPEVKFNWYVDGVEVHNAKTKPREEQYNSTYRVVSVLTVLHQDWLNGKEYKCKVSNKALPAPIEKTISKAKGQPREPQVYTLPPSREEMTKNQVSLTCLVKGFYPSDIAVEWESNGQPENNYKTTPPVLDSDGSFFLYSKLTVDKSRWQQGNVFSCSVMHEALHNHYTQKSLSLSPG

SEQ ID NO: 38 - protein, 107 aa, Artificial Sequence [sequence omitted]

SEQ ID NO: 39 - protein, 446 aa, Artificial Sequence
  900759(Oleclumab) heavy chain sequence
EVQLLESGGGLVQPGGSLRLSCAASGFTFSSYAYSWVRQAPGKGLEWVSAISGSGGRTYYADSVKGRFTISRDNSKNTLYLQMNSLRAEDTAVYYCARLGYGRVDEWGRGTLVTVSSASTKGPSVFPLAPSSKSTSGGTAALGCLVKDYFPEPVTVSWNSGALTSGVHTFPAVLQSSGLYSLSSVVTVPSSSLGTQTYICNVNHKPSNTKVDKRVEPKSCDKTHTCPPCPAPEAAGGPSVFLFPPKPKDTLMISRTPEVTCVVVDVSHEDPEVKFNWYVDGVEVHNAKTKPREEQYNSTYRVVSVLTVLHQDWLNGKEYKCKVSNKALPAPIEKTISKAKGQPREPQVYTLPPSREEMTKNQVSLTCLVKGFYPSDIAVEWESNGQPENNYKTTPPVLDSDGSFFLYSKLTVDKSRWQQGNVFSCSVMHEALHNHYTQKSLSLSPG

SEQ ID NO: 40 - protein, 216 aa, Artificial Sequence
  900759(Oleclumab) light chain sequence
QSVLTQPPSASGTPGQRVTISCSGSLSNIGRNPVNWYQQLPGTAPKLLIYLDNLRLSGVPDRFSGSKSGTSASLAISGLQSEDEADYYCATWDDSHPGWTFGGGTKLTVLGQPKAAPSVTLFPPSSEELQANKATLVCLISDFYPGAVTVAWKADSSPVKAGVETTTPSKQSNNKYAASSYLSLTPEQWKSHRSYSCQVTHEGSTVEKTVAPTECS

SEQ ID NO: 41 - protein, 25 aa, Artificial Sequence
  900567(124A9) H-FR1; H-FR1 of 900725 900726; H-FR1 of 900727 900728
  misc_feature (5)..(5): Xaa = Gln or Val
  misc_feature (7)..(7): Xaa = Pro or Ser
  misc_feature (11)..(11): Xaa = Leu or Val
  misc_feature (12)..(12): Xaa = Lys or Val
  misc_feature (20)..(20): Xaa = Leu or Val
QVQLXQXGAEXXKPGASVKXSCKAS

SEQ ID NO: 42 - protein, 17 aa, Artificial Sequence
  900567(124A9) H-FR2; H-FR2 of 900725 900726 900727 900728
  misc_feature (5)..(5): Xaa = Lys or Arg
  misc_feature (7)..(7): Xaa = Ala or Arg
  misc_feature (13)..(13): Xaa = Asp or Glu
IHWVXQXPGQGLXWIGM

SEQ ID NO: 43 - protein, 38 aa, Artificial Sequence
  900567(124A9) H-FR3; H-FR3 of 900725 900726;900727 H-FR3; 900728 H-FR3
  misc_feature (3)..(3): Xaa = Ala or Asn
  misc_feature (4)..(4): Xaa = Glu or Gln
  misc_feature (7)..(7): Xaa = Lys or Gln
  misc_feature (8)..(8): Xaa = Gly or Ser
  misc_feature (9)..(9): Xaa = Lys or Arg
  misc_feature (10)..(10): Xaa = Ala or Val
  misc_feature (12)..(12): Xaa = Ile or Leu or Met
  misc_feature (18)..(18): Xaa = Ser or Thr
  misc_feature (24)..(24): Xaa = Glu or Gln
  misc_feature (29)..(29): Xaa = Arg or Thr
  misc_feature (33)..(33): Xaa = Ser or Thr
YYXXKFXXXXTXTVDKSXSTAYMXLSSLXSEDXAVYYC

SEQ ID NO: 44 - protein, 11 aa, Artificial Sequence
  900567(124A9) H-FR4; H-FR4 of 900725 900726 900727 900728
  misc_feature (3)..(3): Xaa = Gln or Thr
WGXGTTVTVSS

SEQ ID NO: 45 - protein, 26 aa, Artificial Sequence
  900567(124A9) L-FR1; L-FR1 of 900725 900727;L-FR1 of 900726 900728
  misc_feature (3)..(3): Xaa = Gln or Val
  misc_feature (8)..(8): Xaa = Pro or Gln
  misc_feature (9)..(9): Xaa = Lys or Ser
  misc_feature (10)..(10): Xaa = Phe or Ser
  misc_feature (11)..(11): Xaa = Leu or Met
  misc_feature (13)..(13): Xaa = Ala or Thr
  misc_feature (20)..(20): Xaa = Ser or Thr
DIXMTQSXXXXSXSVGDRVXITCKAS

SEQ ID NO: 46 - protein, 17 aa, Artificial Sequence
  900567(124A9) L-FR2; L-FR2 of 900725 900726 900727 900728
  misc_feature (7)..(7): Xaa = Lys or Asn
  misc_feature (10)..(10): Xaa = Lys or Gln
  misc_feature (11)..(11): Xaa = Ala or Ser
VVWYQQXPGXXPKALIY

SEQ ID NO: 47 - protein, 36 aa, Artificial Sequence
  900567(124A9) L-FR3;L-FR3 of 900725 900727; L-FR3 of 900726 900728
  misc_feature (11)..(11): Xaa = Ser or Thr
  misc_feature (25)..(25): Xaa = Asn or Ser
  misc_feature (26)..(26): Xaa = Leu or Val
  misc_feature (27)..(27): Xaa = His or Gln
  misc_feature (28)..(28): Xaa = Pro or Ser
  misc_feature (31)..(31): Xaa = Phe or Leu
  misc_feature (33)..(33): Xaa = Asp or Thr
  misc_feature (35)..(35): Xaa = Phe or Tyr
NRHTGVPDRFXGSGSGTDFTLTISXXXXEDXAXYXC

SEQ ID NO: 48 - protein, 10 aa, Artificial Sequence
  900567(124A9) L-FR4;  L-FR4 of 900725 900726 900727 900728
  misc_feature (3)..(3): Xaa = Gly or Gln
FGXGTKLEIK

SEQ ID NO: 49 - protein, 121 aa, Artificial Sequence
  900567(124A9) VH; VH of 900725 900726; 900727 VH; 900728 VH
  misc_feature (5)..(5): Xaa = Gln or Val
  misc_feature (7)..(7): Xaa = Pro or Ser
  misc_feature (11)..(11): Xaa = Leu or Val
  misc_feature (12)..(12): Xaa = Lys or Val
  misc_feature (20)..(20): Xaa = Leu or Val
  misc_feature (38)..(38): Xaa = Lys or Arg
  misc_feature (40)..(40): Xaa = Ala or Arg
  misc_feature (46)..(46): Xaa = Asp or Glu
  misc_feature (61)..(61): Xaa = Ala or Asn
  misc_feature (62)..(62): Xaa = Glu or Gln
  misc_feature (65)..(65): Xaa = Lys or Gln
  misc_feature (66)..(66): Xaa = Gly or Ser
  misc_feature (67)..(67): Xaa = Lys or Arg
  misc_feature (68)..(68): Xaa = Ala or Val
  misc_feature (70)..(70): Xaa = Ile or Leu or Met
  misc_feature (76)..(76): Xaa = Ser or Thr
  misc_feature (82)..(82): Xaa = Glu or Gln
  misc_feature (87)..(87): Xaa = Arg or Thr
  misc_feature (91)..(91): Xaa = Ser or Thr
  misc_feature (113)..(113): Xaa = Gln or Thr
QVQLXQXGAEXXKPGASVKXSCKASGYTFTSYWIHWVXQXPGQGLXWIGMIHPNSGSTYYXXKFXXXXTXTVDKSXSTAYMXLSSLXSEDXAVYYCARYYGSDYEWYFDVWGXGTTVTVSS

SEQ ID NO: 50 - protein, 107 aa, Artificial Sequence
  900567(124A9)VL; VL of 900725 900727;VL of 900726 900728
  misc_feature (3)..(3): Xaa = Gln or Val
  misc_feature (8)..(8): Xaa = Pro or Gln
  misc_feature (9)..(9): Xaa = Lys or Ser
  misc_feature (10)..(10): Xaa = Phe or Ser
  misc_feature (11)..(11): Xaa = Leu or Met
  misc_feature (13)..(13): Xaa = Ala or Thr
  misc_feature (20)..(20): Xaa = Ser or Thr
  misc_feature (39)..(39): Xaa = Lys or Asn
  misc_feature (42)..(42): Xaa = Lys or Gln
  misc_feature (43)..(43): Xaa = Ala or Ser
  misc_feature (63)..(63): Xaa = Ser or Thr
  misc_feature (77)..(77): Xaa = Asn or Ser
  misc_feature (78)..(78): Xaa = Leu or Val
  misc_feature (79)..(79): Xaa = His or Gln
  misc_feature (80)..(80): Xaa = Pro or Ser
  misc_feature (83)..(83): Xaa = Phe or Leu
  misc_feature (85)..(85): Xaa = Asp or Thr
  misc_feature (87)..(87): Xaa = Phe or Tyr
  misc_feature (100)..(100): Xaa = Gly or Gln
DIXMTQSXXXXSXSVGDRVXITCKASQNVRTAVVWYQQXPGXXPKALIYLASNRHTGVPDRFXGSGSGTDFTLTISXXXXEDXAXYXCLQHWNYPYTFGXGTKLEIK

SEQ ID NO: 51 - protein, 450 aa, Artificial Sequence
  900201 heavy chain
QIQLVQSGPELKKPGETVKISCKTSGYTFTNYGMNWVKQAPGKGLKWVGWINTYTGEPKYADDFKGRFAFSVETSASTAYLQINNLKNEDTATYFCARGIYDGYHWYFDVWGAGTTVTVSSASTKGPSVFPLAPSSKSTSGGTAALGCLVKDYFPEPVTVSWNSGALTSGVHTFPAVLQSSGLYSLSSVVTVPSSSLGTQTYICNVNHKPSNTKVDKRVEPKSCDKTHTCPPCPAPELLGGPSVFLFPPKPKDTLMISRTPEVTCVVVDVSHEDPEVKFNWYVDGVEVHNAKTKPREEQYNSTYRVVSVLTVLHQDWLNGKEYKCKVSNKALPAPIEKTISKAKGQPREPQVYTLPPSREEMTKNQVSLTCLVKGFYPSDIAVEWESNGQPENNYKTTPPVLDSDGSFFLYSKLTVDKSRWQQGNVFSCSVMHEALHNHYTQKSLSLSPG

SEQ ID NO: 52 - protein, 219 aa, Artificial Sequence
  900201 light chain
DVVMTQTPLSLPVSLGDQASISCRSSQSLVHSIGNTYLHWYLQKPGQSPKLLIYKVSNRFSGVPDRFSGSGSGTDFTLKITRVEAEDLGVYFCSQSTHVPFTFGSGTKLEIKRTVAAPSVFIFPPSDEQLKSGTASVVCLLNNFYPREAKVQWKVDNALQSGNSQESVTEQDSKDSTYSLSSTLTLSKADYEKHKVYACEVTHQGLSSPVTKSFNRGEC

SEQ ID NO: 53 - protein, 447 aa, Artificial Sequence
  Oleclumab heavy chain
EVQLLESGGGLVQPGGSLRLSCAASGFTFSSYAYSWVRQAPGKGLEWVSAISGSGGRTYYADSVKGRFTISRDNSKNTLYLQMNSLRAEDTAVYYCARLGYGRVDEWGRGTLVTVSSASTKGPSVFPLAPSSKSTSGGTAALGCLVKDYFPEPVTVSWNSGALTSGVHTFPAVLQSSGLYSLSSVVTVPSSSLGTQTYICNVNHKPSNTKVDKRVEPKSCDKTHTCPPCPAPEFEGGPSVFLFPPKPKDTLMISRTPEVTCVVVDVSHEDPEVKFNWYVDGVEVHNAKTKPREEQYNSTYRVVSVLTVLHQDWLNGKEYKCKVSNKALPASIEKTISKAKGQPREPQVYTLPPSREEMTKNQVSLTCLVKGFYPSDIAVEWESNGQPENNYKTTPPVLDSDGSFFLYSKLTVDKSRWQQGNVFSCSVMHEALHNHYTQKSLSLSPGK

SEQ ID NO: 54 - protein, 215 aa, Artificial Sequence
  Oleclumab light chain
QSVLTQPPSASGTPGQRVTISCSGSLSNIGRNPVNWYQQLPGTAPKLLIYLDNLRLSGVPDRFSGSKSGTSASLAISGLQSEDEADYYCATWDDSHPGWTFGGGTKLTVLQPKAAPSVTLFPPSSEELQANKATLVCLISDFYPGAVTVAWKADSSPVKAGVETTTPSKQSNNKYAASSYLSLTPEQWKSHRSYSCQVTHEGSTVEKTVAPTECS

SEQ ID NO: 55 - protein, 450 aa, Artificial Sequence
  900543 HC
QIQLVQSGPELKKPGETVKISCKTSGYTFTNYGMNWVKQAPGKGLKWVGWINTYTGEPKYADDFKGRFAFSVETSASTAYLQINNLKNEDTATYFCARGIYDGYHWYFDVWGAGTTVTVSSASTKGPSVFPLAPSSKSTSGGTAALGCLVKDYFPEPVTVSWNSGALTSGVHTFPAVLQSSGLYSLSSVVTVPSSSLGTQTYICNVNHKPSNTKVDKRVEPKSCDKTHTCPPCPAPEAAGGPSVFLFPPKPKDTLMISRTPEVTCVVVDVSHEDPEVKFNWYVDGVEVHNAKTKPREEQYNSTYRVVSVLTVLHQDWLNGKEYKCKVSNKALPAPIEKTISKAKGQPREPQVYTLPPSREEMTKNQVSLTCLVKGFYPSDIAVEWESNGQPENNYKTTPPVLDSDGSFFLYSKLTVDKSRWQQGNVFSCSVMHEALHNHYTQKSLSLSPG